European Patent Application EP 4 471 059 A1, published December 4, 2024. Title: Antibody Molecule Against Growth And Differentiation Factor 15 And Use Thereof. Applicant: Yunnan Baiyao Group Co., Ltd. The sequence listing filed with the application follows.

SEQUENCE LISTING (52 sequences)

SEQ ID NO: 1 - protein, 120 aa, Artificial Sequence
  VH
EVLLQQSGPELVKPGASVKIPCKASGYTFTDYNMDWVKQSHGKSLEWIGQINPNNGGIFFNQKFKGKATLTVDKSSNTAFMEVRSLTSEDTAVYYCAREAITTVGAMDYWGQGTSVTVSS

SEQ ID NO: 2 - protein, 107 aa, Artificial Sequence
  VL
DIQMTQSPASLSASVGETVTITCRTSENLHNYLAWYQQKQGKSPQLLVYDAKTLADGVPSRFSGSGSGTQYSLKINSLQPEDFGSYYCQHFWSSPYTFGGGTKLEIK

SEQ ID NO: 3 - protein, 324 aa, Artificial Sequence
  CH1-CH3
AKTTPPSVYPLAPGSAAQTNSMVTLGCLVKGYFPEPVTVTWNSGSLSSGVHTFPAVLQSDLYTLSSSVTVPSSTWPSETVTCNVAHPASSTKVDKKIVPRDCGCKPCICTVPEVSSVFIFPPKPKDVLTITLTPKVTCVVVDISKDDPEVQFSWFVDDVEVHTAQTQPREEQFNSTFRSVSELPIMHQDWLNGKEFKCRVNSAAFPAPIEKTISKTKGRPKAPQVYTIPPPKEQMAKDKVSLTCMITDFFPEDITVEWQWNGQPAENYKNTQPIMDTDGSYFVYSKLNVQKSNWEAGNTFTCSVLHEGLHNHHTEKSLSHSPGK

SEQ ID NO: 4 - protein, 107 aa, Artificial Sequence
  CL1
RADAAPTVSIFPPSSEQLTSGGASVVCFLNNFYPKDINVKWKIDGSERQNGVLNSWTDQDSKDSTYSMSSTLTLTKDEYERHNSYTCEATHKTSTSPIVKSFNRNEC

SEQ ID NO: 5 - protein, 330 aa, Artificial Sequence [sequence omitted]

SEQ ID NO: 6 - protein, 107 aa, Artificial Sequence [sequence omitted]

SEQ ID NO: 7 - protein, 118 aa, Artificial Sequence
  VH
QVQLKESGPGILQPSQTLSLTCSFSGFSLSTSGMGVGWIRQPSGKGLEWLAHILWDDVKRYNPALKSRLTISKDSSNSQIFLKIASVDTADTATYYCVQMAWDWFAYWGQGTLVTVSA

SEQ ID NO: 8 - protein, 106 aa, Artificial Sequence
  VL
DIVMTQAQKFMSTSVEDRVSVTCKASQNVDTNVAWYQQKPGQSPKALIYSASYRSSGVPDRFTGSGSGTDFTLTISNVQSEDLAEYFCQQYHSYPTFGGGTKLEIK

SEQ ID NO: 9 - protein, 118 aa, Artificial Sequence
  VH
QVQLKESGPGILQPSQTLSLTCSFSGFSLSTSGMGVGWIRQPSGKGLEWLAHIRWDDVKRYNPALKSRLTISKDTSSSQIFLKIASVDTADTATYYCAQMAWDWFAYWGQGTLVTVSA

SEQ ID NO: 10 - protein, 106 aa, Artificial Sequence
  VL
DIVMTQAQKFMSTSVGDRVSVTCKASQNVDTDVAWYQQKPGQSPKALIYSASYRYSGVPDRFTGSGSGTDFTLTITNVQSEDLAEYFCHQYNSYPTFGGGTKLEIK

SEQ ID NO: 11 - protein, 120 aa, Artificial Sequence
  VH
QVQLKESGPGILQPSQTLSLTCSFSGFSLNTAGMTVGWIRQPSGKGLEWLAHIWWNDDKYYNPALKSRLTISKDTSNNQIFLEIASVVTADTATYYCTRIATMNYAMDYWGQGTSVTVSS

SEQ ID NO: 12 - protein, 111 aa, Artificial Sequence
  VL
DIVMTQAPASLAVSLGQRATISCRASQSVSTSSFSYMHWYQQKPGQPPKLLIKYASNLESGVPARFSGSGSGTDFTLNIHPVEEEDTATYYCQHSWEIPYTFGGGTKLEIK

SEQ ID NO: 13 - protein, 118 aa, Artificial Sequence
  VH
QVTLKESGPGILQPSQTLSLTCSFSGFSLTTSGMGVDWIRQSSGKGLEWLAHIYWDDDKRYNPSLKSRLTISKDTSSNQVFLKITSVDTADTATYYCARRAWDAMDYWGQGTSFTVSS

SEQ ID NO: 14 - protein, 107 aa, Artificial Sequence
  VL
DIVMTQAQKFMSTSVGDRVSVTCKARQNVGTNVAWYQQKPGQSPKALIYSASYRYSGVPDRFTGSGSGTDFTLTISNVQSEDLAEYFCQQYNSYPYTFGGGTKLEIK

SEQ ID NO: 15 - protein, 118 aa, Artificial Sequence
  VH
QVTLKESGPGILKPSQTLSLTCSFSGFSLSTSGMGVGWIRQPSGKGLEWLAHIWWNDDKYYNPSLKSHLTISKDTSRNQVFLMITSVDTADTATYYCARGAYDFFDYWGQGTTLTVSS

SEQ ID NO: 16 - protein, 107 aa, Artificial Sequence
  VL
DIVMTQAQNFMSTSVGDRVSVTCKASQNVDTNVAWYQQKPGQSPKALIYSASYRYSGVPDRFTGSGSGTDFTLTISNVQSDDLADYFCQQYNTYPYTFGGGTKLEIK

SEQ ID NO: 17 - protein, 118 aa, Artificial Sequence
  VH
QVTLKESGPGIVQPSQPFRLTCTFSGFSLSTSGIGITWIRQPSGKGLEWLATIWWDDDNRYNPSLKSRLTVSKDTSNNQAFLNIITVETADTAIYYCVQSAWDWFAYWGQGTLVTVSA

SEQ ID NO: 18 - protein, 107 aa, Artificial Sequence
  VL
DIVMTQSQKFMSTSVGDRVSVTCKASQNVGTNVAWYQQKSGQSPKALIYSASYRNSGVPDRFTGSGSGTDFTLTISNVESEDLAEYFCQQYNSHPVTFGGGTKLEIK

SEQ ID NO: 19 - protein, 118 aa, Artificial Sequence
  VH
QVQLQESGPGLVKPSETLSLTCTFSGFSLSTSGMGVGWIRQPPGKGLEWLAHILWDDVKRYNPALKSRLTISKDSSKSQISLKLSSVTAADTAVYYCVQMAWDWFAYWGQGTTVTVSS

SEQ ID NO: 20 - protein, 106 aa, Artificial Sequence
  VL
DIQMTQSPSSLSASVGDRVTITCKASQNVDTNVAWYQQKPGQSPKALIYSASYRSSGVPSRFSGSGSGTDFTLTISSLQPEDFATYYCQQYHSYPTFGQGTRLEIK

SEQ ID NO: 21 - protein, 118 aa, Artificial Sequence
  VH
QVQLQESGPGLVKPSETLSLTCTFSGFSLSTSGMGVGWIRQPPGKGLEWLAHIRWDDVKRYNPALKSRLTISKDTSKSQISLKLSSVTAADTAVYYCAQMAWDWFAYWGQGTTVTVSS

SEQ ID NO: 22 - protein, 106 aa, Artificial Sequence
  VL
DIQMTQSPSSLSASVGDRVTITCKASQNVDTDVAWYQQKPGQSPKALIYSASYRYSGVPSRFSGSGSGTDFTLTISSLQPEDFATYYCHQYNSYPTFGQGTRLEIK

SEQ ID NO: 23 - protein, 7 aa, Artificial Sequence
  HCDR-1
TSGMGVG

SEQ ID NO: 24 - protein, 16 aa, Artificial Sequence
  HCDR-2
HILWDDVKRYNPALKS

SEQ ID NO: 25 - protein, 8 aa, Artificial Sequence
  HCDR-3
MAWDWFAY

SEQ ID NO: 26 - protein, 11 aa, Artificial Sequence
  LCDR-1
KASQNVDTNVA

SEQ ID NO: 27 - protein, 7 aa, Artificial Sequence
  LCDR-2
SASYRSS

SEQ ID NO: 28 - protein, 8 aa, Artificial Sequence
  LCDR-3
QQYHSYPT

SEQ ID NO: 29 - protein, 16 aa, Artificial Sequence
  HCDR-2
HIRWDDVKRYNPALKS

SEQ ID NO: 30 - protein, 11 aa, Artificial Sequence
  LCDR-1
KASQNVDTDVA

SEQ ID NO: 31 - protein, 7 aa, Artificial Sequence
  LCDR-2
SASYRYS

SEQ ID NO: 32 - protein, 8 aa, Artificial Sequence
  LCDR-3
HQYNSYPT

SEQ ID NO: 33 - protein, 7 aa, Artificial Sequence
  HCDR-1
TAGMTVG

SEQ ID NO: 34 - protein, 16 aa, Artificial Sequence
  HCDR-2
HIWWNDDKYYNPALKS

SEQ ID NO: 35 - protein, 10 aa, Artificial Sequence
  HCDR-3
IATMNYAMDY

SEQ ID NO: 36 - protein, 15 aa, Artificial Sequence
  LCDR-1
RASQSVSTSSFSYMH

SEQ ID NO: 37 - protein, 7 aa, Artificial Sequence
  LCDR-2
YASNLES

SEQ ID NO: 38 - protein, 9 aa, Artificial Sequence
  LCDR-3
QHSWEIPYT

SEQ ID NO: 39 - protein, 7 aa, Artificial Sequence
  HCDR-1
TSGMGVD

SEQ ID NO: 40 - protein, 16 aa, Artificial Sequence
  HCDR-2
HIYWDDDKRYNPSLKS

SEQ ID NO: 41 - protein, 8 aa, Artificial Sequence
  HCDR-3
RAWDAMDY

SEQ ID NO: 42 - protein, 11 aa, Artificial Sequence
  LCDR-1
KARQNVGTNVA

SEQ ID NO: 43 - protein, 9 aa, Artificial Sequence
  LCDR-3
QQYNSYPYT

SEQ ID NO: 44 - protein, 16 aa, Artificial Sequence
  HCDR-2
HIWWNDDKYYNPSLKS

SEQ ID NO: 45 - protein, 8 aa, Artificial Sequence
  HCDR-3
GAYDFFDY

SEQ ID NO: 46 - protein, 9 aa, Artificial Sequence
  LCDR-3
QQYNTYPYT

SEQ ID NO: 47 - protein, 7 aa, Artificial Sequence
  HCDR-1
TSGIGIT

SEQ ID NO: 48 - protein, 16 aa, Artificial Sequence
  HCDR-2
TIWWDDDNRYNPSLKS

SEQ ID NO: 49 - protein, 8 aa, Artificial Sequence
  HCDR-3
SAWDWFAY

SEQ ID NO: 50 - protein, 11 aa, Artificial Sequence
  LCDR-1
KASQNVGTNVA

SEQ ID NO: 51 - protein, 7 aa, Artificial Sequence
  LCDR-2
SASYRNS

SEQ ID NO: 52 - protein, 9 aa, Artificial Sequence
  LCDR-3
QQYNSHPVT